European Patent Application EP 4 592 307 A2, published July 30, 2025. Title: A rose bengal-sonosensitiser complex. Applicant: University of Ulster. Application EP EP18734205.0, filed June 25, 2018. The sequence listing filed with the application follows.

SEQUENCE LISTING (6 sequences)

SEQ ID NO: 1 - protein, 14 aa, unidentified
  REGION 1..14: note = Synthetic peptide
KLAKLAKKLAKLAK

SEQ ID NO: 2 - protein, 15 aa, unidentified
  REGION 1..15: note = Synthetic peptide
CKLAKLAKKLAKLAK

SEQ ID NO: 3 - protein, 4 aa, unidentified
  REGION 1..4: note = Synthetic peptide
KLAK

SEQ ID NO: 4 - protein, 29 aa, unidentified
  REGION 1..29: note = Synthetic peptide
CKLAKLAKKLAKLAKKLAKLAKKLAKLAK

SEQ ID NO: 5 - protein, 7 aa, unidentified
  REGION 1..7: note = Synthetic peptide
KLAKLAK

SEQ ID NO: 6 - protein, 8 aa, unidentified
  REGION 1..8: note = Synthetic peptide
CKLAKLAK